European Patent Application EP 4 303 230 A1, published January 10, 2024. Title: Alpha-1 Antitrypsin Dosing Regimen. Applicant: GRIFOLS WORLDWIDE OPERATIONS LIMITED. The sequence listing filed with the application follows.

SEQUENCE LISTING (9 sequences)

SEQ ID NO: 1 - protein, 418 aa, Homo sapiens
MPSSVSWGILLLAGLCCLVPVSLAEDPQGDAAQKTDTSHHDQDHPTFNKITPNLAEFAFSLYRQLAHQSNSTNIFFSPVSIATAFAMLSLGTKADTHDEILEGLNFNLTEIPEAQIHEGFQELLRTLNQPDSQLQLTTGNGLFLSEGLKLVDKFLEDVKKLYHSEAFTVNFGDTEEAKKQINDYVEKGTQGKIVDLVKELDRDTVFALVNYIFFKGKWERPFEVKDTEEEDFHVDQVTTVKVPMMKRLGMFNIQHCKKLSSWVLLMKYLGNATAIFFLPDEGKLQHLENELTHDIITKFLENEDRRSASLHLPKLSITGTYDLKSVLGQLGITKVFSNGADLSGVTEEAPLKLSKAVHKAVLTIDEKGTEAAGAMFLEAIPMSIPPEVKFNKPFVFLMIEQNTKSPLFMGKVVNPTQK

SEQ ID NO: 2 - protein, 679 aa, Homo sapiens
VPDKTVRWCAVSEHEATKCQSFRDHMKSVIPSDGPSVACVKKASYLDCIRAIAANEADAVTLDAGLVYDAYLAPNNLKPVVAEFYGSKEDPQTFYYAVAVVKKDSGFQMNQLRGKKSCHTGLGRSAGWNIPIGLLYCDLPEPRKPLEKAVANFFSGSCAPCADGTDFPQLCQLCPGCGCSTLNQYFGYSGAFKCLKDGAGDVAFVKHSTIFENLANKADRDQYELLCLDNTRKPVDEYKDCHLAQVPSHTVVARSMGGKEDLIWELLNQAQEHFGKDKSKEFQLFSSPHGKDLLFKDSAHGFLKVPPRMDAKMYLGYEYVTAIRNLREGTCPEAPTDECKPVKWCALSHHERLKCDEWSVNSVGKIECVSAETTEDCIAKIMNGEADAMSLDGGFVYIAGKCGLVPVLAENYNKSDNCEDTPEAGYFAVAVVKKSASDLTWDNLKGKKSCHTAVGRTAGWNIPMGLLYNKINHCRFDEFFSEGCAPGSKKDSSLCKLCMGSGLNLCEPNNKEGYYGYTGAFRCLVEKGDVAFVKHQTVPQNTGGKNPDPWAKNLNEKDYELLCLDGTRKPVEEYANCHLARAPNHAVVTRKDKEACVHKILRQQQHLFGSNVTDCSGNFCLFRSETKDLLFRDDTVCLAKLHDRNTYEKYLGEEYVKAVGNLRKCSTSSLLEACTFRRP

SEQ ID NO: 3 - protein, 692 aa, Homo sapiens
GRRRRSVQWCTVSQPEATKCFQWQRNMRRVRGPPVSCIKRDSPIQCIQAIAENRADAVTLDGGFIYEAGLAPYKLRPVAAEVYGTERQPRTHYYAVAVVKKGGSFQLNELQGLKSCHTGLRRTAGWNVPIGTLRPFLNWTGPPEPIEAAVARFFSASCVPGADKGQFPNLCRLCAGTGENKCAFSSQEPYFSYSGAFKCLRDGAGDVAFIRESTVFEDLSDEAERDEYELLCPDNTRKPVDKFKDCHLARVPSHAVVARSVNGKEDAIWNLLRQAQEKFGKDKSPKFQLFGSPSGQKDLLFKDSAIGFSRVPPRIDSGLYLGSGYFTAIQNLRKSEEEVAARRARVVWCAVGEQELRKCNQWSGLSEGSVTCSSASTTEDCIALVLKGEADAMSLDGGYVYTAGKCGLVPVLAENYKSQQSSDPDPNCVDRPVEGYLAVAVVRRSDTSLTWNSVKGKKSCHTAVDRTAGWNIPMGLLFNQTGSCKFDEYFSQSCAPGSDPRSNLCALCIGDEQGENKCVPNSNERYYGYTGAFRCLAENAGDVAFVKDVTVLQNTDGNNNDAWAKDLKLADFALLCLDGKRKPVTEARSCHLAMAPNHAVVSRMDKVERLKQVLLHQQAKFGRNGSDCPDKFCLFQSETKNLLFNDNTECLARLHGKTTYEKYLGPQYVAGITNLKKCSTSPLLEACEFLRK

SEQ ID NO: 4 - protein, 679 aa, Artificial Sequence
  Mutant protein
VPDKTVRWCAVSEHEATKCQSFRDHMKSVIPSDGPSVACVKKASYLDCIRAIAANEADAVTLDAGLVYDAYLAPNNLKPVVAEFYGSKEDPQTFYYAVAVVKKDSGFQMNQLRGKKSCHTGLGRSAGWNIPIGLLYCDLPEPRKPLEKAVANFFSGSCAPCADGTDFPQLCQLCPGCGCSTLNQYFGFSGAFKCLKDGAGDVAFVKHSTIFENLANKADRDQYELLCLDNTRKPVDEYKDCHLAQVPSHTVVARSMGGKEDLIWELLNQAQEHFGKDKSKEFQLFSSPHGKDLLFKDSAHGFLKVPPRMDAKMYLGYEYVTAIRNLREGTCPEAPTDECKPVKWCALSHHERLKCDEWSVNSVGKIECVSAETTEDCIAKIMNGEADAMSLDGGFVYIAGKCGLVPVLAENYNKSDNCEDTPEAGYFAVAVVKKSASDLTWDNLKGKKSCHTAVGRTAGWNIPMGLLYNKINHCRFDEFFSEGCAPGSKKDSSLCKLCMGSGLNLCEPNNKEGYYGYTGAFRCLVEKGDVAFVKHQTVPQNTGGKNPDPWAKNLNEKDYELLCLDGTRKPVEEYANCHLARAPNHAVVTRKDKEACVHKILRQQQHLFGSNVTDCSGNFCLFRSETKDLLFRDDTVCLAKLHDRNTYEKYLGEEYVKAVGNLRKCSTSSLLEACTFRRP

SEQ ID NO: 5 - protein, 679 aa, Artificial Sequence
  Mutant protein
VPDKTVRWCAVSEHEATKCQSFRDHMKSVIPSDGPSVACVKKASYLDCIRAIAANEADAVTLDAGLVYDAYLAPNNLKPVVAEFYGSKEDPQTFFYAVAVVKKDSGFQMNQLRGKKSCHTGLGRSAGWNIPIGLLYCDLPEPRKPLEKAVANFFSGSCAPCADGTDFPQLCQLCPGCGCSTLNQYFGFSGAFKCLKDGAGDVAFVKHSTIFENLANKADRDQYELLCLDNTRKPVDEYKDCHLAQVPSHTVVARSMGGKEDLIWELLNQAQEHFGKDKSKEFQLFSSPHGKDLLFKDSAHGFLKVPPRMDAKMYLGYEYVTAIRNLREGTCPEAPTDECKPVKWCALSHHERLKCDEWSVNSVGKIECVSAETTEDCIAKIMNGEADAMSLDGGFVYIAGKCGLVPVLAENYNKSDNCEDTPEAGYFAVAVVKKSASDLTWDNLKGKKSCHTAVGRTAGWNIPMGLLYNKINHCRFDEFFSEGCAPGSKKDSSLCKLCMGSGLNLCEPNNKEGYYGYTGAFRCLVEKGDVAFVKHQTVPQNTGGKNPDPWAKNLNEKDYELLCLDGTRKPVEEYANCHLARAPNHAVVTRKDKEACVHKILRQQQHLFGSNVTDCSGNFCLFRSETKDLLFRDDTVCLAKLHDRNTYEKYLGEEYVKAVGNLRKCSTSSLLEACTFRRP

SEQ ID NO: 6 - protein, 679 aa, Artificial Sequence
  Mutant protein
VPDKTVRWCAVSEHEATKCQSFRDHMKSVIPSDGPSVACVKKASYLDCIRAIAANEADAVTLDAGLVYDAYLAPNNLKPVVAEFYGSKEDPQTFYYAVAVVKKDSGFQMNQLRGKKSCHTGLGRSAGWNIPIGLLYCDLPEPRKPLEKAVANFFSGSCAPCADGTDFPQLCQLCPGCGCSTLNQYFGYSGAFKCLKDGAGDVAFVKHSTIFENLANKADRDQYELLCLDNTRKPVDEYKDCHLAQVPSHTVVARSMGGKEDLIWELLNQAQEHFGKDKSKEFQLFSSPHGKDLLFKDSAHGFLKVPPRMDAKMYLGYEYVTAIRNLREGTCPEAPTDECKPVKWCALSHHERLKCDEWSVNSVGKIECVSAETTEDCIAKIMNGEADAMSLDGGFVYIAGKCGLVPVLAENYNKSDNCEDTPEAGFFAVAVVKKSASDLTWDNLKGKKSCHTAVGRTAGWNIPMGLLYNKINHCRFDEFFSEGCAPGSKKDSSLCKLCMGSGLNLCEPNNKEGYYGFTGAFRCLVEKGDVAFVKHQTVPQNTGGKNPDPWAKNLNEKDYELLCLDGTRKPVEEYANCHLARAPNHAVVTRKDKEACVHKILRQQQHLFGSNVTDCSGNFCLFRSETKDLLFRDDTVCLAKLHDRNTYEKYLGEEYVKAVGNLRKCSTSSLLEACTFRRP

SEQ ID NO: 7 - protein, 679 aa, Artificial Sequence
  Mutant protein
VPDKTVRWCAVSEHEATKCQSFRDHMKSVIPSDGPSVACVKKASYLDCIRAIAANEADAVTLDAGLVYDAYLAPNNLKPVVAEFYGSKEDPQTFFYAVAVVKKDSGFQMNQLRGKKSCHTGLGRSAGWNIPIGLLYCDLPEPRKPLEKAVANFFSGSCAPCADGTDFPQLCQLCPGCGCSTLNQYFGFSGAFKCLKDGAGDVAFVKHSTIFENLANKADRDQYELLCLDNTRKPVDEYKDCHLAQVPSHTVVARSMGGKEDLIWELLNQAQEHFGKDKSKEFQLFSSPHGKDLLFKDSAHGFLKVPPRMDAKMYLGYEYVTAIRNLREGTCPEAPTDECKPVKWCALSHHERLKCDEWSVNSVGKIECVSAETTEDCIAKIMNGEADAMSLDGGFVYIAGKCGLVPVLAENYNKSDNCEDTPEAGYFAVAVVKKSASDLTWDNLKGKKSCHTAVGRTAGWNIPMGLLYNKINHCRFDEFFSEGCAPGSKKDSSLCKLCMGSGLNLCEPNNKEGYYGFTGAFRCLVEKGDVAFVKHQTVPQNTGGKNPDPWAKNLNEKDYELLCLDGTRKPVEEYANCHLARAPNHAVVTRKDKEACVHKILRQQQHLFGSNVTDCSGNFCLFRSETKDLLFRDDTVCLAKLHDRNTYEKYLGEEYVKAVGNLRKCSTSSLLEACTFRRP

SEQ ID NO: 8 - protein, 679 aa, Artificial Sequence
  Mutant protein
VPDKTVRWCAVSEHEATKCQSFRDHMKSVIPSDGPSVACVKKASYLDCIRAIAANEADAVTLDAGLVYDAYLAPNNLKPVVAEFYGSKEDPQTFFYAVAVVKKDSGFQMNQLRGKKSCHTGLGRSAGWNIPIGLLYCDLPEPRKPLEKAVANFFSGSCAPCADGTDFPQLCQLCPGCGCSTLNQYFGFSGAFKCLKDGAGDVAFVKHSTIFENLANKADRDQYELLCLDNTRKPVDEYKDCHLAQVPSHTVVARSMGGKEDLIWELLNQAQEHFGKDKSKEFQLFSSPHGKDLLFKDSAHGFLKVPPRMDAKMYLGYEYVTAIRNLREGTCPEAPTDECKPVKWCALSHHERLKCDEWSVNSVGKIECVSAETTEDCIAKIMNGEADAMSLDGGFVYIAGKCGLVPVLAENYNKSDNCEDTPEAGFFAVAVVKKSASDLTWDNLKGKKSCHTAVGRTAGWNIPMGLLYNKINHCRFDEFFSEGCAPGSKKDSSLCKLCMGSGLNLCEPNNKEGYYGFTGAFRCLVEKGDVAFVKHQTVPQNTGGKNPDPWAKNLNEKDYELLCLDGTRKPVEEYANCHLARAPNHAVVTRKDKEACVHKILRQQQHLFGSNVTDCSGNFCLFRSETKDLLFRDDTVCLAKLHDRNTYEKYLGEEYVKAVGNLRKCSTSSLLEACTFRRP

SEQ ID NO: 9 - protein, 906 aa, Artificial Sequence
  Mutant protein
VPDKTVRWCAVSEHEATKCQSFRDHMKSVIPSDGPSVACVKKASYLDCIRAIAANEADAVTLDAGLVYDAYLAPNNLKPVVAEFYGSKEDPQTFFYAVAVVKKDSGFQMNQLRGKKSCHTGLGRSAGWNIPIGLLYCDLPEPRKPLEKAVANFFSGSCAPCADGTDFPQLCQLCPGCGCSTLNQYFGFSGAFKCLKDGAGDVAFVKHSTIFENLANKADRDQYELLCLDNTRKPVDEYKDCHLAQVPSHTVVARSMGGKEDLIWELLNQAQEHFGKDKSKEFQLFSSPHGKDLLFKDSAHGFLKVPPRMDAKMYLGYEYVTAIRNLREGTCPEAPTDECKPVKWCALSHHERLKCDEWSVNSVGKIECVSAETTEDCIAKIMNGEADAMSLDGGFVYIAGKCGLVPVLAENYNKSDNCEDTPEAGFFAVAVVKKSASDLTWDNLKGKKSCHTAVGRTAGWNIPMGLLYNKINHCRFDEFFSEGCAPGSKKDSSLCKLCMGSGLNLCEPNNKEGYYGFTGAFRCLVEKGDVAFVKHQTVPQNTGGKNPDPWAKNLNEKDYELLCLDGTRKPVEEYANCHLARAPNHAVVTRKDKEACVHKILRQQQHLFGSNVTDCSGNFCLFRSETKDLLFRDDTVCLAKLHDRNTYEKYLGEEYVKAVGNLRKCSTSSLLEACTFRRPDKTHTCPPCPAPELLGGPSVFLFPPKPKDTLMISRTPEVTCVVVDVSHEDPEVKFNWYVDGVEVHNAKTKPREEQYNSTYRVVSVLTVLHQDWLNGKEYKCKVSNKALPAPIEKTISKAKGQPREPQVYTLPPSRDELTKNQVSLTCLVKGFYPSDIAVEWESNGQPENNYKTTPPVLDSDGSFFLYSKLTVDKSRWQQGNVFSCSVMHEALHNHYTQKSLSLSPGK